European Patent Specification EP 3 068 439 B1, published June 26, 2024. Title: OLIGOPEPTIDES AND METHODS FOR PRODUCING CONJUGATES THEREOF. Applicant: F. HOFFMANN-LA ROCHE INSTITUT PASTEUR CENTRE NATIONAL DE LA RECHERCHE SCIENTIFIQUE COMMISSARIAT A L'ENERGIE ATOMIQUE ET AUX ENERGIES ALTERNATIVES. The sequence listing filed with the application follows.

SEQUENCE LISTING (18 sequences)

SEQ ID NO: 1 - protein, 13 aa, Artificial Sequence
  CDR1 of VHH R3VE/Q
ADSGSTFRNYNIG

SEQ ID NO: 2 - protein, 17 aa, Artificial Sequence
  CDR2 of VHH R3VE/Q
AVSRTGISTHVADSLQG

SEQ ID NO: 3 - protein, 18 aa, Artificial Sequence
  CDR3 of VHH R3VE/Q
AAGRPGVGAVNRAMDYDY

SEQ ID NO: 4 - protein, 127 aa, Lama pacos
MAEVQLQASGGGLVQTGDSLRLSCADSGSTFRNYNIGWFRQTPGQAREFVAAVSRTGISTHVADSLQGRFTISRDNAKNTVYLQMNSLKPEDTAVYSCAAGRPGVGAVNRAMDYDYWGQGTQVTVSS

SEQ ID NO: 5 - protein, 127 aa, Lama pacos
MAEVQLEASGGGLVQTGDSLRLSCADSGSTFRNYNIGWFRQTPGQAREFVAAVSRTGISTHVADSLQGRFTISRDNAKNTVYLQMNSLKPEDTAVYSCAAGRPGVGAVNRAMDYDYWGQGTQVTVSS

SEQ ID NO: 6 - protein, 122 aa, Lama pacos
VQLQASGGGLVQTGDSLRLSCADSGSTFRNYNIGWFRQTPGQAREFVAAVSRTGISTHVADSLQGRFTISRDNAKNTVYLQMNSLKPEDTAVYSCAAGRPGVGAVNRAMDYDYWGQGTQVTV

SEQ ID NO: 7 - protein, 122 aa, Lama pacos
VQLEASGGGLVQTGDSLRLSCADSGSTFRNYNIGWFRQTPGQAREFVAAVSRTGISTHVADSLQGRFTISRDNAKNTVYLQMNSLKPEDTAVYSCAAGRPGVGAVNRAMDYDYWGQGTQVTV

SEQ ID NO: 8 - protein, 151 aa, Artificial Sequence
  R3VQ-SH
  DOMAIN (5)..(6): 6xHis tag
  DOMAIN (14)..(19): Thrombin cleavage site
  DOMAIN (23)..(144): VHH R3VQ
  DOMAIN (145)..(148): Spacer
  DOMAIN (150)..(151): Spacer
MGSSHHHHHHSSGLVPRGSAAAVQLQASGGGLVQTGDSLRLSCADSGSTFRNYNIGWFRQTPGQAREFVAAVSRTGISTHVADSLQGRFTISRDNAKNTVYLQMNSLKPEDTAVYSCAAGRPGVGAVNRAMDYDYWGQGTQVTVGGGSCSA

SEQ ID NO: 9 - protein, 6 aa, Artificial Sequence
  6xHis tag
HHHHHH

SEQ ID NO: 10 - protein, 6 aa, Artificial Sequence
  Thrombin cleavage site
LVPRGS

SEQ ID NO: 11 - protein, 4 aa, Artificial Sequence
  Spacer
GGGS

SEQ ID NO: 12 - protein, 42 aa, Artificial Sequence [sequence omitted]

SEQ ID NO: 13 - DNA, 41 bp, Artificial Sequence
  Primer
ggactagttgcggccgctggttgtggttttggtgtcttggg

SEQ ID NO: 14 - protein, 123 aa, Lama pacos
MAEVQLQASGGGLVQAGGSRRLSCAVSGRTFSSYNMGWFRQAPGEEREFVAAINWSASTYYADSVKGRFTISRDNAKNTVYLQMNSLKPEDTAVYYCNLHVATTSYFQTSDYWGQGTQVTVSS

SEQ ID NO: 15 - protein, 123 aa, Lama pacos
MAEVQLQASGGGLVQAGGSLRLSCAVSGRTFSSYNMGWFRQAPGKEREFVAAINWSASTYYADSVKGRFTISRDNAKNTVYLQMNSLKPEDTAVYYCNLHVATTSYFQTSDYWGQGTQVTVSS

SEQ ID NO: 16 - protein, 124 aa, Lama pacos
MADVQLQASGGGLVQPGGSLELSCAASGSTFSINVMGWYRQSPDGVRDLVATITANGVTNYAASVKGRFTISKDNAKNTVFLQMNSVKPEDTAVYICNVEGEYSGSYVADFDSWGQGTQVTVSS

SEQ ID NO: 17 - DNA, 465 bp, Artificial Sequence
  Nucleotide sequence encoding R3VQ-SH
atgggcagcagccatcatcatcatcatcacagcagcggcctggtgccgcgcggcagcgcggccgcagtccagctgcaggcgtctggaggaggattggtgcagactggggactctctgagactctcctgtgcagactctggaagtacattcagaaactataacataggctggttccgccagactccaggacaggcgcgtgaatttgtcgcagctgttagtcggacgggaattagcacacacgttgcagactccctccagggccgattcaccatctccagagacaacgccaagaacacggtgtatctgcaaatgaacagcctgaaacctgaggacacggccgtttattcctgtgcagcggggcgaccgggcgtaggagctgtcaacagggcgatggattatgactactggggccaggggacccaggtcaccgtcggtggcggatcctgttccgcgtaataactcgag

SEQ ID NO: 18 - protein, 152 aa, Artificial Sequence
  VHH R3VE-SH
  misc_feature (98)..(98): Xaa can be any naturally occurring amino acid
MGSSHHHHHHSSGLVPRGSAAAEVQLEASGGGLVQTGDSLRLSCADSGSTFRNYNIGWFRQTPGQAREFVAAVSRTGISTHVADSLQGRFTISRDNAXNTVYLQMNSLKPEDTAVYSCAAGRPGVGAVNRAMDYDYWGQGTQVTVGGGSCSA